European Patent Specification EP 3 919 520 B1, published July 10, 2024. Title: ANTIBODY AND FUNCTIONAL FRAGMENT THEREOF. Applicant: SUMITOMO CHEMICAL COMPANY, LIMITED. The sequence listing filed with the application follows.

SEQUENCE LISTING (14 sequences)

SEQ ID NO: 1 - protein, 8 aa, Mus musculus
GIDFSIYW

SEQ ID NO: 2 - protein, 8 aa, Mus musculus
INSDSSTI

SEQ ID NO: 3 - protein, 13 aa, Mus musculus
ARKNGGLDYAMDY

SEQ ID NO: 4 - protein, 6 aa, Mus musculus
KSISKY

SEQ ID NO: 5 - protein, 9 aa, Mus musculus
QQHNEYPWT

SEQ ID NO: 6 - DNA, 24 bp, Mus musculus
ggaatcgattttagtatatactgg

SEQ ID NO: 7 - DNA, 24 bp, Mus musculus
attaattcagatagcagtacaata

SEQ ID NO: 8 - DNA, 39 bp, Mus musculus
gcaagaaagaatgggggattggactatgctatggactac

SEQ ID NO: 9 - DNA, 18 bp, Mus musculus
aagagcattagcaaatat

SEQ ID NO: 10 - DNA, 27 bp, Mus musculus
caacagcataatgaatacccgtggacg

SEQ ID NO: 11 - protein, 138 aa, Mus musculus
MDFGLIFFIVALLKGVQCEVKLLQSGGGLVQPGGSLKLSCAASGIDFSIYWMSWVRRAPGKGLEWIGEINSDSSTINYAPSLKDKFTISRDNAKNTLYLQMSKVRSEDTALYYCARKNGGLDYAMDYWGQGTSVTVSS

SEQ ID NO: 12 - protein, 122 aa, Mus musculus
MVLISLLFWISGAQCDVQITQSPSYLAASPGETITINCRSSKSISKYLAWYQEKPGKTNKLLIYSGSTLQSGIPSRFSGSGSGTDFTLTISSLEPEDFAMYYCQQHNEYPWTFGGGTKLEIK

SEQ ID NO: 13 - DNA, 414 bp, Mus musculus
atggattttgggctgattttttttattgttgctcttttaaaaggggtccagtgtgaggtgaagcttctccagtctggaggtggcctggtgcagcctggaggatccctgaaactctcctgtgcagcctcaggaatcgattttagtatatactggatgagttgggttcggcgggctccagggaaaggactagaatggattggagaaattaattcagatagcagtacaataaactatgcaccatctctaaaggataaattcaccatctccagagacaacgccaaaaatacgctgtacctgcaaatgagcaaagtgagatctgaggacacagccctttattactgtgcaagaaagaatgggggattggactatgctatggactactggggtcaaggaacctcagtcaccgtctcctca

SEQ ID NO: 14 - DNA, 366 bp, Mus musculus
atggttctcatatccttgctgttctggatatcaggtgcccagtgtgatgtccagataacccagtctccatcttatcttgctgcatctcctggagaaaccattactattaattgcaggtcaagtaagagcattagcaaatatttagcctggtatcaagagaaacctgggaaaactaataagcttcttatctactctggatccactttacaatctggaattccatcaaggttcagtggcagtggatctggtacagatttcactctcaccatcagtagcctggagcctgaagattttgcaatgtattactgtcaacagcataatgaatacccgtggacgttcggtggaggcaccaagctggaaatcaag